European Patent Specification EP 3 993 826 B1, published April 29, 2026. Title: NOVEL CANCER ANTIGENS AND METHODS. Applicant: The Francis Crick Institute Limited Enara Bio Limited. The sequence listing filed with the application follows.

SEQUENCE LISTING (39 sequences)

SEQ ID NO: 1 - protein, 83 aa, Homo sapiens [sequence omitted]

SEQ ID NO: 2 - protein, 84 aa, Homo sapiens
MWNSLEARSPKSRCCSTGPWEAVQENLLWASLLAPGGATIFPDPWLLKASPSSLPHLHRTSPCACLCPNFPFYKDTVLLHQGPR

SEQ ID NO: 3 - protein, 77 aa, Homo sapiens [sequence omitted]

SEQ ID NO: 4 - protein, 43 aa, Homo sapiens
MIVRPPQPCGTKCLRITSGVKVKKKTVNCVLTALKNEKSCQAK

SEQ ID NO: 5 - protein, 59 aa, Homo sapiens
MSPPGGRNNSRHAALRAVTLTAKVCSFTPEPVRPRTRHKEETLNTSSEHQKEQTPDAPP

SEQ ID NO: 6 - protein, 38 aa, Homo sapiens
MCALQGRGASPAGAGLFHWTMSPFLLGSLYGHIHNEAV

SEQ ID NO: 7 - protein, 55 aa, Homo sapiens
MRFGDLSSLLKALTLKDFMKLKFKSRCAPSKDHPLYTATCCFPWIKKHKEPSSTT

SEQ ID NO: 8 - protein, 59 aa, Homo sapiens [sequence omitted]

SEQ ID NO: 9 - protein, 9 aa, Homo sapiens
GLNSIIWRL

SEQ ID NO: 10 - protein, 10 aa, Homo sapiens
ILIQTTGIFK

SEQ ID NO: 11 - protein, 11 aa, Homo sapiens
ATIFPDPWLLK

SEQ ID NO: 12 - protein, 9 aa, Homo sapiens
FPFYKDTVL

SEQ ID NO: 13 - protein, 10 aa, Homo sapiens
FPFYKDTVLL

SEQ ID NO: 14 - protein, 10 aa, Homo sapiens
TIFPDPWLLK

SEQ ID NO: 15 - protein, 9 aa, Homo sapiens
IVLDAPVTK

SEQ ID NO: 16 - protein, 9 aa, Homo sapiens
RITSGVKVK

SEQ ID NO: 17 - protein, 10 aa, Homo sapiens
RITSGVKVKK

SEQ ID NO: 18 - protein, 10 aa, Homo sapiens
ALRAVTLTAK

SEQ ID NO: 19 - protein, 8 aa, Homo sapiens
GHIHNEAV

SEQ ID NO: 20 - protein, 11 aa, Homo sapiens
SLYGHIHNEAV

SEQ ID NO: 21 - protein, 11 aa, Homo sapiens
APSKDHPLYTA

SEQ ID NO: 22 - protein, 9 aa, Homo sapiens
RLFSEDIHV

SEQ ID NO: 23 - DNA, 2749 bp, Homo sapiens
gtttttgccatctgtagtgttgcccttagcaacagaaaagcatgtgacagtgcttatgtgactctgctggcctgcaacagtgtgtagaaggatttaagcaaaatgaaacagacagaaatattgatccagacaactggaattttcaagtgtattgcaatgataatgacgactggaaaggaaagagaggaaggtaacaaagaaaagccaagaaaactatttggagtgagagactatggtaatataaaaggctataatgtggtaaaatcgtggggacttaattccatcatatggaggttactgaatgtatcagagacagcctgcagttcatcaccacacaaattaggagcaacgtaagaagagaaaaagaaaaaggaattacagattaaaaaatgcaagagaatataaacaaataaaaatatgttcaactggaatttgtattgggattgtattaaatggatgaactaatttgtgaagaaatgatatcattccatccaagagcatggaactcctatttttcctattgtcttctatgtttctttttaaaaagtcttaagttttctctgtagagttttttgcattctggatgattttaattgaaacatactgtatagatattgttactatgataagtggtgcctcttattagattttttaattcattatgattggtaaagcaaataggaaagattttgagcatagaaaactgcctcaattacctcattacttcaaaaagtattgccattggttctattgctttttaaaaaaatacatgatgatatcttctgcacattatgaaattttatctcaacactttcaatcaccgcatctctgtttgacactgatgaacatttccaaagtgaaatattttgctctctttatttttctccttttgctctttggggcctctttactttctaaacttgtcacttcttggtttatcttccaaacctcttggcttttcttttgtgtagtatactttagcttcattctgggagagtttttcattctgaacttttcgattcactagtttattctccatcagtatgtatgctaatttttcttccattgactttttttcccaaacacttatttttcatactttatattttcacttggaattttgggggaatattttgttctagtttcaaattgatcctatattttttgtctccttaagtatatttatcaggcttattttaaattcttgatttatatgttataataatgctaccttagatggcatatgctgctcaatttttctttcctttttccactctagtagtggtagtcctctggcttctggttatttttgtctctagagttatgttatgttattataacagatgtgagaaagggcccaaaaccaggttttagcctgtgtctgctctaatgagttaatgtgattactctggatgatcttcagagtagaatacaataagcaattgttgtttattacaagtttcgaatttgtaactgtgaaatctactgtgcttcctaatttagcacctttaacaatctatgatctaggctattgcttccaacttttaaagtttaagggaaaacattgattgtcccaaggaaatgtggtcagaggaaataacagaggtaatactcaaaataagaaatactcaaaataagttaatgtgaaaaataatagtatagaagcagctcaagaaggaaatgatgagttgcaaggtcagattgaagaactgttccagaaggcagcaagaaacaataatgtaaaatttttaaaattaataataataacaaaaaactaaaagacatggaggatagaaatagatatatatggtgtgttgtatgagatgagtcagttaacttatgagcaagcaacccaaccatatctaaacatatacctgagtatgctttaactcatgtacttacaaaattgcatttcttagtgaaaaaaaaatcaagaaagaaaacaattcctaaggttagtgatgaaagtataaagtcaagagataaactagtgattttcaaaaaaaaaaaaaagtaactttagagtggcaaatcaaatgtcactctgttcatacaagattcatgaaactgtttcagagagggttttgttccttgcaaaagttgttcacccacaagagacagattttgtaaaatttaaaatgtagctaattttccatgtgattaggcagtgtaatttaaagaaactcaagattttctacaaataattttttgaggcaagaagatgctaaagtcacttgtactgccactaaactttactaaaagttggtttgaacactttaattgcttttgaatagatgattgaagctgtgaagaggtggcagcagctgacatgttgccatggtagcatttcctccccagctgaggaggctatacagaagaaaggatataggtcagaaagtgtttatactgacaaaacaaccacatattaaaatcaaatgcttttgtaaacatcataagccaaatgagagttgtgaaatctagtttcaggatattaaagacagactgatttatctttaggatgatgtatcaagctgtactgtgagaatggagcattcaaggtcaagaatactctccttcctgcatattggcaattcaattttaaaagattgaaacacgatgaaagtgtttctatcagtttcttctgtgttccttgcaataaggatatatttaattgaaaaattcttcttgaaggtagttcatctctgaataaactactccagggtaaggaagatcaactctatgatcaata

SEQ ID NO: 24 - DNA, 3103 bp, Homo sapiens
gaggcctcacagccatgtggaactctctggaggccagaagtccaaaatcaagatgttgcagcactggtccctgggaggctgtgcaggagaatctgctctgggcgtctctcctggctcctggtggtgccacaatcttccctgatccttggcttttgaaggcatcccccagctctctgcctcatcttcacaggacttctccctgtgcctgtctgtgcccaaatttccccttctataaggacacagtcctactgcatcagggcccacgctaatcacttcttcttcactaattacatcggcaaaccccctatttccaagttaagtcatgttctgaggttaggatttcaatacctgaattttaggggacatagttcagcccaaaggacctggggggacagaaacacccaggaaagtccacaggtcagcgcctggacccgcctggccgtgggacattgctcggccgagttcatcctcataaacgctgacgtgtgctagaagatacaatattagtttcataaacaacagtttctttttttgcaaaccatacccacaggtcctattgccacttttcagtgctgcagcagctagtcagatgacaactgggtgagagcttggtctcgagtgtttcctgtgaggccagaatattgctctgattcctcaggggtgactcagccctccggtgggaaatatgtgacctcatttgcatttcctaattgaattgctatcagctttcctgcaagactgcaccaaaaaacagttcttccagattccagcactgcctgcattgcccacagaaaggctgcttttaaatagttgctaagagagggcgacaaaagaaggagaaaagttgccaaatttttatggttcatctaactgtaaagctgtcagttttacccagctccccagagtcgctaaaataatggacagaggaggcggcacttgaagaaacctcgacataagagaaatgaaatttacagaaccaggaaattaggggtccccatgcacctgccctggcagaatctgcttccaggctcctctcaataaacactgccctgggactcccagcgctctgtaaactgatgctttgaaggaggccatttgtttctccagaaccttctgccagcagaactcttgcttaccacgtgcccccatcagaactcccaccttctctaaacacagttaggtagccctctgcatgcatttgtttaaaaaaattaaattgtgagtaatagactataagtacaacagcgtacagaacaccagctaaaaaaatgatggcagaatgagcacctgtcttgccacaagactccctcccaccctctggtgtcccccagcatggcttcctgctgccccctgaaaggaaccctcaaccgactgtaactctgcacctcagtgccacccgaatttggacttcatgggagtgcggtcactcggctgacacgtgttcctgctgccaggcacctgcctgctctccttctttggtctgtttgtgagattcgctggctttgttgcttctagctgcagtttgttcacttttactgccgtataatattccactttaggagcccactgcaatttattgactcattgcaatggtgagggcatgtgtgttgtttccagcttttggtgattatgcgtaagatttctcttaacgtcccgtacagagttcttggtattacctgcctatactgctatgggcatacaccaaaaacgaggcatatgtatatttgactttaatagtaattctgaattgctgtctaaagtgtttgtaccattgtacactcccatcaagagtatacgagtgctgcaaatgtcctttcccagactctgccttattgtctcatttttaagatatatgttttgatgatcagaagttctttttttttttttttttttttgacaggcttttgctctgttgcccaggctggagtgcagtggcatgatctcagctcactgcaacctctacctctcgggctcaagtgattctcctgtttgagactccctagtagctgggattacaggtgtgcaccaccatgcctagctaatttttgtatttttagtggagacagggtttcaccatgttagccaggctggtctcgaactcctgaccttgggtgatctgcccaccttggcctcccaaagtgctgggattacaggcgtgagccaccgcacctggcagaagttcttatttttaataaagtccagtgatcattctttcccgtgtttcacgcttcacgtgccatgtgcgaggaagctttccacacccgggggtcagttcactcccagctgcattgctttgcctttcctgtttaggttttcagtccacctcaaatggattttggttgtggtgtgaggtaggggtcattttacttttttcttaaagatgccccattggcccagcatcatttattgaaaagacagtctttcctctgttgtttctgtagaaatgggcaaactttcccccaaatggccagatggtaaatattttaggcatctcaggttaaggggcaaaattgaggacatcgtataggtacttacataaccctttaaaatggaaccatttaaaaatgtaaaaaccagtcttagcttgctggccataaaaggcctgtgggctacagcatgctggcacctgctctacagcactgctcttataataaaaaatcaagcgtctgcaccctgggcatttgacaaggctcatcagattgtaaagatgaactgggtggattttgtagtatgagagttatacgtccatgaagctgatttttaaacacattacatgtctttttctgggctcattatttttgttccaagtgtctatctaatcatctttgcttcaaaatgacaccgttttaatggctgtagttcagtggttctcaaaagggggcagttttgccccccagggaacatttggcagtggctggaaagagctttggttgcatatggaggttatggggctttacctggcgtttagtgggtagaggccaggagtctggcttactatcctgtagcacacaggacagccccaacaacttgtctggaaggatgtgtcctcccatctttttcttgttctaggctaccttcgccctttccatttccattaaaaaat

SEQ ID NO: 25 - DNA, 1907 bp, Homo sapiens
gtgtgccctttgcagcaaagagcgtggttcctcctcttcctgggtgtaaactgcgattcaaaaagccaggtgggaagccctgtagtagggactctggctttgtccctgtttcccccttttcttcctcttcacccactaaaaccctgttttactcacggttcaaattgtttggcagcctgaattttcatggccatgggacaaagaaccccgtctttagctgaattaaggaaaagttctgcaacatttttgacgtgcaacttgggggctcaagcggagaagcgaagcagagcccctggaaaactcacatatgtgtcaacaatagtccttgatgcccctgtaacaaaacttgagcaaggcctggtgatgaagagatacaagattgtcacccaaggatttgattatacctctgttgaaagttaatgcacactcaaccgaatatggcaattggtactctcaattctatattctcaacaattacagtgaagatacaagtagaatacaatcactgccacattttttgaaattctgtgtaaactgtaatattctgtcaacattaatgacatttgaagtgtcctgtcaaaacaattgcagctactttatgtataaaacatattaaataggctcatccaacttgcattctttattaagcttattttcatattttttcctatggatgaacttaaaaataattttgtttcttaattaagattctatgcatgaagatgctgaataatttaagacaattgttcattcaaatagttgctaattacaccctcctggcatagttattgtattattactacatttaggaataatatgctgtactacttggacttgaaaatgtttctgacattttaatgaacacactacttagttatattttacaagggttttcagtgaaccacagaggattaaaaaatgtcattcaagggttgtagataattaaactgactgaatataagaagcctcatatggaagtgaaaattatgtatgaattttgttgagctggaaatgtgttttactaaatgacttcagatttgttacttttaaatacaagatgaagggaatcaaggggatactttcttctcacctcaatttgttccatttgcataagctattttatctttcaatatcccttttgatatttcattttggcccttgaatacactaaagattatttaaaataaataaatgttgactttgaaatactgctatatatattcattgcaatacatcaggtgggaaattggtgcaattcagtcacacacacaacctcatagatcagatttccagttaagttttaatagaaagagattttagatagacatgactttcaataaaatggaagaatttttattagtttcaaaataatgattttacttgcttatcaacacagttgacctttccccacagtactatgatcttcttagtacctctgctataattatattaatgtcttcctatatctagaaatttgattattattctatttttatggatcattaaatttttctattcaagaatgatccctatagtcaacttcctgagggatttctgcttgctattttctgtttcaattgtgtgcatttcatatttactattaaagattttaaataatgacacattgtttaagcggttgtaagtctgattgttataaagctctctggagaattctgtaagctttcacatctgatggagaacttcaatgagaacatctttaatgtggaattcttggacaagaaactacagattatccatggttcagaagatatgatgaattagtaactatttttccgtacataaaaagtcaatcttcctaaccagtttgttgttttagctaaatgaatcggtcaaatattttagttatattagcaatattttgtctctaaaatatcttgacataaaac

SEQ ID NO: 26 - DNA, 327 bp, Homo sapiens
tttgcatttctttcattttccaccatgattgtgaggcctccccagccatgtggaactaaatgcctaagaattacatcaggagtaaaagtgaagaaaaagactgtaaactgcgtgctaactgctttgaagaatgagaagtcatgccaagcaaaatagtagataattgcaagaaggggactaatggtccatggatggagctggaggccattatctttagcaaactaacagaggaacagaaaaccaagtgagaaccacatgttctcacttataagtgggagctaaatgatgagaacacatggacacatagagggaaacaacagacactgg

SEQ ID NO: 27 - DNA, 765 bp, Homo sapiens
ggtagtcacatgtttagcttttaaagaaattgccaaactgtcagagtggctgtcccattttactttccaccagcaatgtatgagtgatttgtcttttcttcatccttagcagcatttgggggctattttttatttcagccgttcttacaagtccacgctgcttttatgagctgtaacactcactgcgaagatctgcagcttcactcctgagcccagcgagaccatgagcccaccgggaggaaggaacaactccagacatgctgccttaagagctgtaacactcactgcgaaggtctgcagcttcactcctgagccagtgagaccacgaacccgccacaaggaagaaactctgaacacatcatctgaacatcagaaggaacaaactccagacgcgccaccttaacagctgtaacactcaccgcgagggtccgcggcttcattcttgaagtcagtgagaccaagaacccaccaattccggacacaccaggaccttccgctgctcgctcctcctcgtcccttctacccgctggggtcagcctcatcgaccccgtctcaactctgacacagtctctctctctctctctctctctatatatatatatatatattttttttttagatggagtctcgctttgctccccaggctggagtgcagtggtgcaatctctgctcactgcaagctccacctcctggtttcacgccattctcctgcctcagcgtcccaagtagctgggactacaggcgcccgccaccacaccctgctaa

SEQ ID NO: 28 - DNA, 3091 bp, Homo sapiens
gggtccctggctcggctctacccccatggatctaggtgaggacaggcgctcctgctttcccgcccaaatgttgtattttccaagcctacccttgccggccacgcccccaacctgggcctataaaaaccgccccccgcaggccctagcgggcagacacactgaagtcgctagacatttgaggaacacatccggggaagaagacacaggtggctggtcatggagagcccgctgggggaagagcacacagacaggcaccggcaggccattgaccagcgggacaaggtggagtttggctggggcagtgggaggagagctggggccgccgagctgccctactccaggggaaaaccacctcccttctcgctcccccatcaccggagagctacttccactcaatacaactttgcactcattctccaagccacgtgtgaccaatttttccggtacaccaaggcgagaaatccggggatacagaaagccctctgtccttgcgataaggtagagggtccaattgagctaacacaagctgcctatagacggcaaactaagagagcacccagtaacacacgcctgctggggcttcaggagcacacacgtccactggggcttcgggagctgtaaacagtcagccctagacactgtcgtgggatcggagccccacagcctgcctgtctgtatgctcctctagaggtctgagcagcggggcgctgaagaaacgagccacactcccatcacacgccctgagaggaggacaagggaacccgtaccgtttcacttgtgatagagataaagttattattgttgtaattttaacttatagaactataatataatggtacaatgatatatattgacaatattcctctttcacccacattttgtatctgtgttcaagattaaatgaaaaaggatattctcaaaaagctagcaaaaccaaaagcaagacgttatgccaaatgtaaacatatttctgtttagcaaatagcaggagtgtataaaacatttctcttttcacataacagaatgttctatgcttactgtattagttaacaaattcaagtctgtttattttgtttgaaattccacttcatccataaattacagcattacacaataacaccagaaggacaatatcaccattgtttgcttttacagtcatctcagcccacaaaatgcttcccattgtcagcttgctatcatcaagctattgttgttttcctctttctggggtcttgtattaatatcattcaaattatttagacactcaacagtgtttttgctatcagtgcaaacctctaaagagctggagccccagcgtgatgaccaaataacccttgactatttatcttgccgtaagtcattatttcctgaggccctggagaagctgtgttgccatgtgtgcactgcagggacggggagcttctcctgccggagctggtttgttccactggacaatgagcccttttctgcttggctctctgtatgggcacatacacaatgaggcggtttagggaagaggggtgatgtgggtcattgataacaacaatccccgaacttcttaaagaattgttgagccccctaaaaatatgttgtctttatgaattatccttaaccctttttaattgcataaaaacttcaggcacttgaaaaaaattaaaaaacgaaaagtaagtctgtctctagtatccctcttctcctttgtagaattacatcctttattcactctgccactatttattatgtgcctcctgtgtgtaagacatactgttagtcattggaaatacagaaatgaatgggacagacacacttcttgccctcatggaacttagggcctaatgggagatacaatgttaaggttgtttctagtgtttttttttttttttaagaatatgttctacatgtatacatgtaatatgtattctctcccatttttaaaaaacataaatggtggtttactatgtgtacgctttttggttttgcattattcttttaacagtatgtagaggatgcattttctactgtatagtgttctgtcccccttaaatagcactctgattttattttgggggggaatcacgactttctaattttgcatactccttgtgggattgtaaatcaggtcccctgtcctcaagtagccaatggttaggtatgcaacccagcttatctctctttagactcaatctcaagcagatccagagttactcaggatcagaacaatatttgaaaggcattaccagaatccagacaagatgatggagcaatacctgatgcccagtggtctagggtagccgattcctgttctgctctccaggctcctgtccattctgtggatcaactcatattgctccaattcattttgttttgcttgcataagccagaattaacttctgttgcttgtaaacaaagagagttaaccaaagacatacagtatatcagagtatagagacctactttactctcggtcattgcctgcatgagtcttctttatatggatgtatcacagtttatttaaccactcccttgtaagtggacatttaagtctagtgttctgtaaataaaaggtcagaatatacgtctgtatacagtatatattcttgcatatccacctttggacagatgtgtgaatgtgttttgtagaaatacatttgtagaaatgcaactgctgggtcaaagaattagtagatttttaataacatcaaacagcgttgaaggcccccatataagaataacaactactgactgaagacataactaattaaaaaaattaattacagcttatttgtaataacttcttattgtcactgagtgaaaaggtaattctcgttgaatttacgaaaagtgactaataggaaatttagaaaactcagagaatatataaaaacacaaagaaaagccagccaccaagtcgcttataattctctcaccaacagtggcagaattacatttagtcatcatcattattcttacatccagttttatagttatttttgaagaggattattatcaactatcaactctgtcatagctggaagtagaggccactaaaacagatttcttaaactccaagtactgtatatggattttctac

SEQ ID NO: 29 - DNA, 1840 bp, Homo sapiens
agagtacttctcagaagtgaatgtcaacttcctgatgtttatactcaaggagaatgaggtttggagatctgagtagtttactgaaggcactcacattgaaagattttatgaagctgaaattcaaatctagatgtgccccatccaaagaccaccctctttatacagcaacatgctgcttcccctggatcaagaaacacaaggagccttcatctaccacataagaattgcagcaaaccctgcagctatcctgaagctgccatgctgaaaaggccaattgggagaccacatagagaccgagagagacttccaaggactccagccaatcctgggccccagcagtttgaatctcccagcaatgccaccatacaggagagggagcaaatactcagaagattcaagtgccagctgcatgggttgatacctacataaaaggcattggcattattcacaagagccaagatatggaaataacctgtgtccattgacagacgaatagatgagggaaacgtggcatatacacacagtggaatattattcggaattaaaaaaagaaggaaatcctgaatcctgctatttctgacaacatgagactgcaggacgttatgaaaatggccacatcatgctcttctagaactttctcatccctcagtcaagaggtggagcctatttacccttgaccttgaaattgatcaggactttgtcactgccttgctcttaacatcaccatgctggagaaatagcatggcaaggccagctggtgatagagaaagatgcctaaggagctccagctgctattttccctggatttttgagtcttcccagtccagccagacatatgactgggcaaaaccctcaggtaactacagccttatccactgtctgactatcacaaaatgagagaccttgggtgaggaccacctacctgagcccagtcatcctgcagagatgcgagaaaaataagaatgtcattattgttattttaaaatcactgagtttgggttaatttgtatgcagcaatagataactgggacacaaagatagactgtaaaaaaataaagagggaatggttaagctaaaaacattgtgatcaaatcaatgtttagtaagtaagcaagaaagatggctatccagggaagagagattgcacaacaaaatgaaaatgaaacaagcaaagaaacaaagcatggattataacttgtaagagagaaaaccatattaaggggagttatttgaatattttgtatgaaaatacagaaatcagatataagtgagctgacactgactttggaggcaggaggaaaactgatggggaattctgggaaaacagaatgatacaaagcagaatcctcaatgtccctacccaaaacctaatgaaataaacagaaatcagcaacattattttaaaaattaattctccaagaacaatacaaaagtaaatggagcaaaaattattattcattttgaaaaagataatctagaaacagagagacagaggaatctagaaaatagtacacaaattcttgtctgagaagtgtctgagaagacatctataggcaaaactgcataaaattctctccagtttggaaggccatcctgggtaattttataaaatgtctctttcataatagaagcctcttcccaacatcatagatgaaaaatttttcaacgaagggaaaatctgttagtgctcatcaatcttcccctacacctcaaggatgagggagtagaggcatagattgagcacaactaattatttccagtaataaacaacatcaagataagacaaagtcttgaggcaatttggttgtcccttgacaaagggaataatgtgaaaggaggt

SEQ ID NO: 30 - DNA, 1319 bp, Homo sapiens
tggtcacctgacattcctgttaggaagaggcctctcctgcccagctcatgtctgcagctacccactgtaacaaaaccacatggaaaaatgagcttgaactggacccctaccttttaccagagaaaaaaagtcaatttgagatgaaacaaagactttaatataagacctaaaactataaaatgtcatataagaaaacctagagaatacccttcttgacgtcagctttggcaaataattcataactaagtcctcaaaagcaatttcaaccaaaagaaaaatggataagttggacctgattaaattaaagggtttctgcacaataaaagaaactatcaacagggtaaacagacagagagaaaatatttgcaaactatgcatccaacagagatctaatatccactatctctaagaaacttgaacaaatcaacaagcaaaagatgaacagccctgttaagaagtgggcaaaaaacatgaacaggctcttctcagaagacatacatgtcgccaacaaacatatgaaaaactactcaaaatcacaagtcaggaaagaaatgcgaatgaaagccataatgaagtaccatcacacaccagtcagaatggctactattaaaaagtaaaaaaataacagatgttgacagggttgtggagaaaagggaatgcgtgttcattattggtgggaatgtaaactatttcagtgcctgtggaacgaaacttggagatatctcaaagaacttacaaaagaacgacgattcgacccagcaattccattactggctttatatccaaaggaaaataaattattctaccaaaaagacacatacattcatatgttcatcaaaacactattcacattaatgaggacatggaatcaatgtagatgtccatcagctatggactggataaagaaaatgtggtacaaacataacatggaatactatgcagccataaaatgaaagaaattatgtactttgcatcaatatggatccagctggagaccattatcttaagtgaattaatgtgggcacagaaagcccaatactgcatgctctcacttataagtgggaactaaacattggttatgcatggacataaagatgggcacaatagacactgggatctaccatgtgggggagggcaggatggagaaagggcctgaagaactgcctattggatattgtgttctctacattggtgttgggattatttgtaccccatacatgagtgtcacacaatatactcatgcaacaaactcacacatgtaccctctggacctaaaataaaagttgaaatgaaaaagagttggtaaatcagtaggtggg

SEQ ID NO: 31 - DNA, 252 bp, Homo sapiens
atgaaacagacagaaatattgatccagacaactggaattttcaagtgtattgcaatgataatgacgactggaaaggaaagagaggaaggtaacaaagaaaagccaagaaaactatttggagtgagagactatggtaatataaaaggctataatgtggtaaaatcgtggggacttaattccatcatatggaggttactgaatgtatcagagacagcctgcagttcatcaccacacaaattaggagcaacgtaa

SEQ ID NO: 32 - DNA, 255 bp, Homo sapiens
atgtggaactctctggaggccagaagtccaaaatcaagatgttgcagcactggtccctgggaggctgtgcaggagaatctgctctgggcgtctctcctggctcctggtggtgccacaatcttccctgatccttggcttttgaaggcatcccccagctctctgcctcatcttcacaggacttctccctgtgcctgtctgtgcccaaatttccccttctataaggacacagtcctactgcatcagggcccacgctaa

SEQ ID NO: 33 - DNA, 234 bp, Homo sapiens
atggccatgggacaaagaaccccgtctttagctgaattaaggaaaagttctgcaacatttttgacgtgcaacttgggggctcaagcggagaagcgaagcagagcccctggaaaactcacatatgtgtcaacaatagtccttgatgcccctgtaacaaaacttgagcaaggcctggtgatgaagagatacaagattgtcacccaaggatttgattatacctctgttgaaagttaa

SEQ ID NO: 34 - DNA, 132 bp, Homo sapiens
atgattgtgaggcctccccagccatgtggaactaaatgcctaagaattacatcaggagtaaaagtgaagaaaaagactgtaaactgcgtgctaactgctttgaagaatgagaagtcatgccaagcaaaatag

SEQ ID NO: 35 - DNA, 180 bp, Homo sapiens
atgagcccaccgggaggaaggaacaactccagacatgctgccttaagagctgtaacactcactgcgaaggtctgcagcttcactcctgagccagtgagaccacgaacccgccacaaggaagaaactctgaacacatcatctgaacatcagaaggaacaaactccagacgcgccaccttaa

SEQ ID NO: 36 - DNA, 117 bp, Homo sapiens
atgtgtgcactgcagggacggggagcttctcctgccggagctggtttgttccactggacaatgagcccttttctgcttggctctctgtatgggcacatacacaatgaggcggtttag

SEQ ID NO: 37 - DNA, 168 bp, Homo sapiens
atgaggtttggagatctgagtagtttactgaaggcactcacattgaaagattttatgaagctgaaattcaaatctagatgtgccccatccaaagaccaccctctttatacagcaacatgctgcttcccctggatcaagaaacacaaggagccttcatctaccacataa

SEQ ID NO: 38 - DNA, 180 bp, Homo sapiens
atgaacagccctgttaagaagtgggcaaaaaacatgaacaggctcttctcagaagacatacatgtcgccaacaaacatatgaaaaactactcaaaatcacaagtcaggaaagaaatgcgaatgaaagccataatgaagtaccatcacacaccagtcagaatggctactattaaaaagtaa

SEQ ID NO: 39 - protein, 10 aa, Homo sapiens
SLYGHIHNEA